European Patent Application EP 4 660 308 A1, published December 10, 2025. Title: Helper Gene. Applicant: 株式会社シンプロジェン. The sequence listing filed with the application follows.

SEQUENCE LISTING (68 sequences)

SEQ ID NO: 1 - DNA, 20 bp, synthetic construct
  misc_feature 1..20: note = primer
  source 1..20: mol_type = other DNA
catcaatgggcgtggatagc

SEQ ID NO: 2 - DNA, 24 bp, synthetic construct
  misc_feature 1..24: note = primer
  source 1..24: mol_type = other DNA
ggagttgttacgacattttggaaa

SEQ ID NO: 3 - DNA, 52 bp, synthetic construct
  misc_feature 1..52: note = primer
  source 1..52: mol_type = other DNA
ttagtaagcttccctcctgacgcggtaggaggaggggagggtgccctgcatg

SEQ ID NO: 4 - DNA, 52 bp, synthetic construct; identical to SEQ ID NO: 3
  misc_feature 1..52: note = primer
  source 1..52: mol_type = other DNA

SEQ ID NO: 5 - DNA, 32 bp, synthetic construct
  misc_feature 1..32: note = primer
  source 1..32: mol_type = other DNA
ccctgcagggaattctaagatacattgatgag

SEQ ID NO: 6 - DNA, 31 bp, synthetic construct
  misc_feature 1..31: note = primer
  source 1..31: mol_type = other DNA
ggaggatccaacttgtttattgcagcttata

SEQ ID NO: 7 - DNA, 33 bp, synthetic construct
  misc_feature 1..33: note = primer
  source 1..33: mol_type = other DNA
caagttggatcctccccagcatgcctgctattc

SEQ ID NO: 8 - DNA, 33 bp, synthetic construct
  misc_feature 1..33: note = primer
  source 1..33: mol_type = other DNA
ttggctagctgtacactgtgccttctagttgcc

SEQ ID NO: 9 - DNA, 33 bp, synthetic construct; identical to SEQ ID NO: 7
  misc_feature 1..33: note = primer
  source 1..33: mol_type = other DNA

SEQ ID NO: 10 - DNA, 60 bp, synthetic construct
  misc_feature 1..60: note = primer
  source 1..60: mol_type = other DNA
gctggccttttgctcgcggccgcagatctacgcgtcctaggctcgacattgattattgac

SEQ ID NO: 11 - DNA, 36 bp, synthetic construct
  misc_feature 1..36: note = primer
  source 1..36: mol_type = other DNA
caatgtcgagcctaggggctccggtgcccgtcagtg

SEQ ID NO: 12 - DNA, 41 bp, synthetic construct
  misc_feature 1..41: note = primer
  source 1..41: mol_type = other DNA
gaagagcggtaccggcgcgcctcacgacacctgaaatggaa

SEQ ID NO: 13 - DNA, 35 bp, synthetic construct
  misc_feature 1..35: note = primer
  source 1..35: mol_type = other DNA
ccggtaccgctcttcgggtggcatccctgtgaccc

SEQ ID NO: 14 - DNA, 35 bp, synthetic construct
  misc_feature 1..35: note = primer
  source 1..35: mol_type = other DNA
tctacgcgtgtcgacaaggacagggaagggagcag

SEQ ID NO: 15 - DNA, 52 bp, synthetic construct
  misc_feature 1..52: note = primer
  source 1..52: mol_type = other DNA
agagctgaagagccctgcaggatggcggcggccggcggggagcgccagctag

SEQ ID NO: 16 - DNA, 46 bp, synthetic construct
  misc_feature 1..46: note = primer
  source 1..46: mol_type = other DNA
atgtatcttagaattcttaatagacaatgaccacgttcggatcgcg

SEQ ID NO: 17 - DNA, 46 bp, synthetic construct
  misc_feature 1..46: note = primer
  source 1..46: mol_type = other DNA
gaaggcacagtgtacatcaggcaaacagaaacgacatcttgtcgtc

SEQ ID NO: 18 - DNA, 46 bp, synthetic construct
  misc_feature 1..46: note = primer
  source 1..46: mol_type = other DNA
caaagaattggctagcatggacaccgcagatatcgtgtgggtggag

SEQ ID NO: 19 - DNA, 47 bp, synthetic construct
  misc_feature 1..47: note = primer
  source 1..47: mol_type = other DNA
gtgtcgtgaggcgcgccatggggcaggaagacgggaaccgcggggag

SEQ ID NO: 20 - DNA, 60 bp, synthetic construct
  misc_feature 1..60: note = primer
  source 1..60: mol_type = other DNA
gccacccgaagagcggtacctcaagacgacggttgagaggtgctgcagggaacggacggc

SEQ ID NO: 21 - DNA, 51 bp, synthetic construct
  misc_feature 1..51: note = primer
  source 1..51: mol_type = other DNA
agagctgaagagccctgcaggatgacggattcccctggcggtgtggccccc

SEQ ID NO: 22 - DNA, 46 bp, synthetic construct
  misc_feature 1..46: note = primer
  source 1..46: mol_type = other DNA
atgtatcttagaattctcaggggaatccaaaaccatacggggtttg

SEQ ID NO: 23 - DNA, 50 bp, synthetic construct
  misc_feature 1..50: note = primer
  source 1..50: mol_type = other DNA
gaaggcacagtgtacatcacagcatatccaacgtcaggtctccctttttg

SEQ ID NO: 24 - DNA, 46 bp, synthetic construct
  misc_feature 1..46: note = primer
  source 1..46: mol_type = other DNA
caaagaattggctagcatggagacaaagcccaagacggcaaccacc

SEQ ID NO: 25 - DNA, 50 bp, synthetic construct; identical to SEQ ID NO: 23
  misc_feature 1..50: note = primer
  source 1..50: mol_type = other DNA

SEQ ID NO: 26 - DNA, 46 bp, synthetic construct; identical to SEQ ID NO: 24
  misc_feature 1..46: note = primer
  source 1..46: mol_type = other DNA

SEQ ID NO: 27 - DNA, 56 bp, synthetic construct
  misc_feature 1..56: note = primer
  source 1..56: mol_type = other DNA
agagctgaagagccctgcaggatgtcgatgacggcctcgtcatccacaccgcggcc

SEQ ID NO: 28 - DNA, 47 bp, synthetic construct
  misc_feature 1..47: note = primer
  source 1..47: mol_type = other DNA
atgtatcttagaattctcaaaaaataagcgtggtgcgtttgtctttg

SEQ ID NO: 29 - DNA, 46 bp, synthetic construct
  misc_feature 1..46: note = primer
  source 1..46: mol_type = other DNA
gaaggcacagtgtacattaagcgttgagccggaaaaaccgcaggcc

SEQ ID NO: 30 - DNA, 46 bp, synthetic construct
  misc_feature 1..46: note = primer
  source 1..46: mol_type = other DNA
caaagaattggctagcatgaccgctcagccgccgctgcaccaccgc

SEQ ID NO: 31 - DNA, 48 bp, synthetic construct
  misc_feature 1..48: note = primer
  source 1..48: mol_type = other DNA
gtgtcgtgaggcgcgccatgacgctcgttctgttcgcaacagagtatg

SEQ ID NO: 32 - DNA, 50 bp, synthetic construct
  misc_feature 1..50: note = primer
  source 1..50: mol_type = other DNA
gccacccgaagagcggtacctcagacggcggtcgccggcggcatgggcgc

SEQ ID NO: 33 - DNA, 52 bp, synthetic construct
  misc_feature 1..52: note = primer
  source 1..52: mol_type = other DNA
agagctgaagagccctgcaggatggatcgcaagacgcgcctctcggagccac

SEQ ID NO: 34 - DNA, 46 bp, synthetic construct
  misc_feature 1..46: note = primer
  source 1..46: mol_type = other DNA
atgtatcttagaattcctagccgcacttttgcttcttggtgttagg

SEQ ID NO: 35 - DNA, 47 bp, synthetic construct
  misc_feature 1..47: note = primer
  source 1..47: mol_type = other DNA
gaaggcacagtgtacattacaaccggctgcgtttggccggcaataac

SEQ ID NO: 36 - DNA, 46 bp, synthetic construct
  misc_feature 1..46: note = primer
  source 1..46: mol_type = other DNA
caaagaattggctagcatgagccacgaggaactaaccgcgctagcg

SEQ ID NO: 37 - DNA, 55 bp, synthetic construct
  misc_feature 1..55: note = primer
  source 1..55: mol_type = other DNA
gtgtcgtgaggcgcgccatgtttttcaacccgtatctgagcggcggcgtgaccgg

SEQ ID NO: 38 - DNA, 51 bp, synthetic construct
  misc_feature 1..51: note = primer
  source 1..51: mol_type = other DNA
gccacccgaagagcggtacctcaacagcattcgtgcgccttgacactgtac

SEQ ID NO: 39 - DNA, 67 bp, synthetic construct
  misc_feature 1..67: note = primer
  source 1..67: mol_type = other DNA
cgaaaagtgccacctgcggccgcaagctttctagaactagtcctaggggctccggtgcccgtcagtg

SEQ ID NO: 40 - DNA, 40 bp, synthetic construct
  misc_feature 1..40: note = primer
  source 1..40: mol_type = other DNA
gctggccttttgctcgcggccgcagatctacgcgtgtcga

SEQ ID NO: 41 - DNA, 49 bp, synthetic construct
  misc_feature 1..49: note = primer
  source 1..49: mol_type = other DNA
atccgaattcgctagcatggatctgcctactaccgtcgtgcgaaaatac

SEQ ID NO: 42 - DNA, 60 bp, synthetic construct
  misc_feature 1..60: note = primer
  source 1..60: mol_type = other DNA
gccacccgaagagcggtaccttaatcgtcgaaaaacgccgcgatcgaggcggcggcgatc

SEQ ID NO: 43 - DNA, 52 bp, synthetic construct; identical to SEQ ID NO: 3
  misc_feature 1..52: note = primer
  source 1..52: mol_type = other DNA

SEQ ID NO: 44 - DNA, 56 bp, synthetic construct
  misc_feature 1..56: note = primer
  source 1..56: mol_type = other DNA
ccttttgctcacatgtcaattggtagatgtacctggacatccaggtgatgccggcg

SEQ ID NO: 45 - DNA, 60 bp, synthetic construct
  misc_feature 1..60: note = primer
  source 1..60: mol_type = other DNA
tgtacaggcgcgccgaattcgttttagggcggagtaacttgtatgtgttgggaattgtag

SEQ ID NO: 46 - DNA, 51 bp, synthetic construct
  misc_feature 1..51: note = primer
  source 1..51: mol_type = other DNA
agggaagcttactaaacggtacacaggaaacaggagacacaactccaagtg

SEQ ID NO: 47 - DNA, 76 bp, synthetic construct
  misc_feature 1..76: note = primer
  source 1..76: mol_type = other DNA
gaaaagtgccacctgacgtcgcggccgcgcgatcgcggtacccaactccatgctcaacagtccccaggtacagccc

SEQ ID NO: 48 - DNA, 60 bp, synthetic construct
  misc_feature 1..60: note = primer
  source 1..60: mol_type = other DNA
gaattcggcgcgcctgtacagcccgggcgaccgcaccctgtgacgaaagccgcccgcaag

SEQ ID NO: 49 - DNA, 108 bp, synthetic construct
  misc_feature 1..108: note = primer
  source 1..108: mol_type = other DNA
gaaaagtgccacctgacgtcgcggccgcggaggggtggagtcgtgacgtgaattacgtcatagggttagggaggtcctgtattagaggtcacgtgagtgttttgcgac

SEQ ID NO: 50 - DNA, 99 bp, synthetic construct
  misc_feature 1..99: note = primer
  source 1..99: mol_type = other DNA
gttcaaacctcccgcttcaaaatggagaccctgcgtgctcactcgggcttaaatacccagcgtgaccacatggtgtcgcaaaatgtcgcaaaacactca

SEQ ID NO: 51 - DNA, 41 bp, synthetic construct
  misc_feature 1..41: note = primer
  source 1..41: mol_type = other DNA
gcgggaggtttgaacgcgcagccgccatgccggggttttac

SEQ ID NO: 52 - DNA, 38 bp, synthetic construct
  misc_feature 1..38: note = primer
  source 1..38: mol_type = other DNA
gatcgcagcgctatttaaatcatttattgttcaaagat

SEQ ID NO: 53 - DNA, 32 bp, synthetic construct
  misc_feature 1..32: note = primer
  source 1..32: mol_type = other DNA
aatagcgctgcgatcgcggcctccaaaaaagc

SEQ ID NO: 54 - DNA, 37 bp, synthetic construct
  misc_feature 1..37: note = primer
  source 1..37: mol_type = other DNA
ccttttgctcacatgtcaattgatcccgcccctaact

SEQ ID NO: 55 - DNA, 23 bp, synthetic construct
  misc_feature 1..23: note = primer
  source 1..23: mol_type = other DNA
aacaataaatgatttaaatcagg

SEQ ID NO: 56 - DNA, 38 bp, synthetic construct
  misc_feature 1..38: note = primer
  source 1..38: mol_type = other DNA
ggccgcgatcgcagcgctgtagccatggaaactagata

SEQ ID NO: 57 - DNA, 31 bp, synthetic construct
  misc_feature 1..31: note = primer
  source 1..31: mol_type = other DNA
tcaccatcttgtcgacacagtcgttgaaggg

SEQ ID NO: 58 - DNA, 44 bp, synthetic construct
  misc_feature 1..44: note = primer
  source 1..44: mol_type = other DNA
agcgcagcgagtcggccggccgcggccgcggaggggtggagtcg

SEQ ID NO: 59 - DNA, 40 bp, synthetic construct
  source 1..40: mol_type = other DNA
  misc_feature 1..40: note = primer
acatctacggattacgtcgaggaggggtggagtcgtgacg

SEQ ID NO: 60 - DNA, 40 bp, synthetic construct
  source 1..40: mol_type = other DNA
  misc_feature 1..40: note = primer
accgcattaaagctcgtcgaagcgctgtagccatggaaac

SEQ ID NO: 61 - DNA, 52 bp, synthetic construct
  source 1..52: mol_type = other DNA
  misc_feature 1..52: note = primer
gtgagcaaaagggcgatcgctctagaactagtgtagccatggaaactagata

SEQ ID NO: 62 - DNA, 22 bp, synthetic construct
  source 1..22: mol_type = other DNA
  misc_feature 1..22: note = primer
caacgactgtgtcgacaagatg

SEQ ID NO: 63 - DNA, 54 bp, synthetic construct
  source 1..54: mol_type = other DNA
  misc_feature 1..54: note = primer
gaaaagtgccacctgcggccgcaagctttctaggcgttacataacttacggtaa

SEQ ID NO: 64 - DNA, 48 bp, synthetic construct
  source 1..48: mol_type = other DNA
  misc_feature 1..48: note = primer
ggtaccggcgcgccggatccgctcttcagctctgcttatatagacctc

SEQ ID NO: 65 - DNA, 48 bp, synthetic construct; identical to SEQ ID NO: 64
  source 1..48: mol_type = other DNA
  misc_feature 1..48: note = primer

SEQ ID NO: 66 - DNA, 61 bp, synthetic construct
  source 1..61: mol_type = other DNA
  misc_feature 1..61: note = primer
gctggccttttgctcgcggccgcagatctacgcgtgtcgacaaggacagggaagggagcag

SEQ ID NO: 67 - DNA, 62 bp, synthetic construct
  source 1..62: mol_type = other DNA
  misc_feature 1..62: note = primer
gctgaagagcggatccgccaccatggacagctcccatctgcgcgatgttgtcatcaagctcc

SEQ ID NO: 68 - DNA, 59 bp, synthetic construct
  source 1..59: mol_type = other DNA
  misc_feature 1..59: note = primer
agcggtaccggcgcgcctacggcatctcgatccagcatatctcctcgtttcgcgggttg